European Patent Specification EP 3 741 844 B1, published November 19, 2025. Title: Production Method of Corneal Endothelial Cell Substitute from iPS cells. Applicant: Keio University. The sequence listing filed with the application follows.

SEQUENCE LISTING (28 sequences)

SEQ ID NO: 1 - DNA, 20 bp, Artificial Sequence
  Forward Primer for OCT 4
gaaacccacactgcagcaga

SEQ ID NO: 2 - DNA, 18 bp, Artificial Sequence
  Reverse Primer for OCT 4
tcgcttgcccttctggcg

SEQ ID NO: 3 - DNA, 21 bp, Artificial Sequence
  Forward Primer for KLF4
tgcggcaaaacctacacaaag

SEQ ID NO: 4 - DNA, 20 bp, Artificial Sequence
  Reverse Primer for KLF4
gggcgaatttccatccacag

SEQ ID NO: 5 - DNA, 20 bp, Artificial Sequence
  Forward Primer for C-MYC
ggacccgcttctctgaaagg

SEQ ID NO: 6 - DNA, 20 bp, Artificial Sequence
  Reverse Primer for C-MYC
taacgttgaggggcatcgtc

SEQ ID NO: 7 - DNA, 19 bp, Artificial Sequence
  Forward Primer for SOX2
gcgccctgcagtacaactc

SEQ ID NO: 8 - DNA, 19 bp, Artificial Sequence
  Reverse Primer for SOX2
cggacttgaccaccgaacc

SEQ ID NO: 9 - DNA, 18 bp, Artificial Sequence
  Forward Primer for SOX9
aacgccttcatggtgtgg

SEQ ID NO: 10 - DNA, 21 bp, Artificial Sequence
  Reverse Primer for SOX9
tctcgctctcgttcagaagtc

SEQ ID NO: 11 - DNA, 19 bp, Artificial Sequence
  Forward Primer for LIN28A
tccgaaccaaccctttgcc

SEQ ID NO: 12 - DNA, 20 bp, Artificial Sequence
  Reverse Primer for LIN28A
caaactgctggttggacacg

SEQ ID NO: 13 - DNA, 21 bp, Artificial Sequence
  Forward Primer for PITX2
ctcctgagagccgaaaagagg

SEQ ID NO: 14 - DNA, 21 bp, Artificial Sequence
  Reverse Primer for PITX2
attcttcccctgctggctttt

SEQ ID NO: 15 - DNA, 20 bp, Artificial Sequence
  Forward Primer for C-JUN
gagctggagcgcctgataat

SEQ ID NO: 16 - DNA, 20 bp, Artificial Sequence
  Reverse Primer for C-JUN
ccctcctgctcatctgtcac

SEQ ID NO: 17 - DNA, 20 bp, Artificial Sequence
  Forward Primer for C-FOS
tactaccactcacccgcaga

SEQ ID NO: 18 - DNA, 20 bp, Artificial Sequence
  Reverse Primer for C-FOS
cgtgggaatgaagttggcac

SEQ ID NO: 19 - DNA, 22 bp, Artificial Sequence
  Forward Primer for NR3C2
tgagctggagatcgtacaaaca

SEQ ID NO: 20 - DNA, 20 bp, Artificial Sequence
  Reverse Primer for NR3C2
gtgcatcccctggcatagtt

SEQ ID NO: 21 - DNA, 20 bp, Artificial Sequence
  Forward Primer for SGK1
gcctgccgcctttttatagc

SEQ ID NO: 22 - DNA, 20 bp, Artificial Sequence
  Reverse Primer for SGK1
caggaggtgtcttgcggaat

SEQ ID NO: 23 - DNA, 20 bp, Artificial Sequence
  Forward Primer for ATP1A1
ccaaagacagggtgctatcg

SEQ ID NO: 24 - DNA, 20 bp, Artificial Sequence
  Reverse Primer for ATP1A1
ttgcttggacacatctgagc

SEQ ID NO: 25 - DNA, 20 bp, Artificial Sequence
  Forward Primer for ITGA3
ggtgcctacaactggaaagg

SEQ ID NO: 26 - DNA, 20 bp, Artificial Sequence
  Reverse Primer for ITGA3
gcctacctgcatcgtgtacc

SEQ ID NO: 27 - DNA, 20 bp, Artificial Sequence
  Forward Primer for ADRB2
ttttggcaacttctggtgcg

SEQ ID NO: 28 - DNA, 20 bp, Artificial Sequence
  Reverse Primer for ADRB2
gatcacgcacagggtctcaa